European Patent Specification EP 3 766 980 B1, published August 7, 2024. Title: Mouse Artificial Chromosome Vector and Its Use. Applicant: National University Corporation Tottori University Trans Chromosomics, Inc. The sequence listing filed with the application follows.

SEQUENCE LISTING (127 sequences)

SEQ ID NO: 1 - DNA, 14 bp, Artificial
  primer
aattcggcgcgccg

SEQ ID NO: 2 - DNA, 40 bp, Artificial
  primer
tcgaggcgcgccagccttctagggaacaggagatgttcaa

SEQ ID NO: 3 - DNA, 38 bp, Artificial
  primer
tcgaggatccgccttgagtggggttctagtcatctttc

SEQ ID NO: 4 - DNA, 28 bp, Artificial
  primer
aactacccagttctgcatttggtgtgag

SEQ ID NO: 5 - DNA, 28 bp, Artificial
  primer
atcagtcatcagtacccccaacctctct

SEQ ID NO: 6 - DNA, 24 bp, Artificial
  primer
gagctgcaagaactcttcctcacg

SEQ ID NO: 7 - DNA, 21 bp, Artificial
  primer
tggatgggtttcaatgccact

SEQ ID NO: 8 - DNA, 20 bp, Artificial
  primer
ggcattctcccctgttgtgg

SEQ ID NO: 9 - DNA, 20 bp, Artificial
  primer
acccctcgaacccctattgc

SEQ ID NO: 10 - DNA, 20 bp, Artificial
  primer
cacgccatcggtgatggata

SEQ ID NO: 11 - DNA, 21 bp, Artificial
  primer
tgggatgacccccacttcttt

SEQ ID NO: 12 - DNA, 20 bp, Artificial
  primer
ttttggcctcttgccccata

SEQ ID NO: 13 - DNA, 38 bp, Artificial
  primer
tcgaggtacctctaagtcagggaaagatccccttcttg

SEQ ID NO: 14 - DNA, 38 bp, Artificial
  primer
tcgactcgaggaccatgaagatggtccaactaaagcaa

SEQ ID NO: 15 - DNA, 40 bp, Artificial
  primer
tcgagtcgaccactgctctttctttagttacatgcagccc

SEQ ID NO: 16 - DNA, 40 bp, Artificial
  primer
tcgagcggccgcattcttgccaagctactcttccgagcta

SEQ ID NO: 17 - DNA, 28 bp, Artificial
  primer
tgagaaataccgaatggcagagaaacac

SEQ ID NO: 18 - DNA, 20 bp, Artificial
  primer
cctgaagttcatctgcacca

SEQ ID NO: 19 - DNA, 26 bp, Artificial
  primer
catcgccttctatcgccttcttgacg

SEQ ID NO: 20 - DNA, 28 bp, Artificial
  primer
gagaggagggaagcttgatgagaaaatg

SEQ ID NO: 21 - DNA, 22 bp, Artificial
  primer
tggaggccataaacaagaagac

SEQ ID NO: 22 - DNA, 21 bp, Artificial
  primer
ccccttgacccagaaattcca

SEQ ID NO: 23 - DNA, 38 bp, Artificial
  primer
tcgaggatccgggagtaattttcaatccttgaggcaga

SEQ ID NO: 24 - DNA, 38 bp, Artificial
  primer
tcgaagatctcatcagtgtacaccacaatcccatctgt

SEQ ID NO: 25 - DNA, 28 bp, Artificial
  primer
cctcttcttgacggttaccacattttgc

SEQ ID NO: 26 - DNA, 21 bp, Artificial
  primer
tgaattggtccctcctgctca

SEQ ID NO: 27 - DNA, 20 bp, Artificial
  primer
caggccatgagacccagaca

SEQ ID NO: 28 - DNA, 20 bp, Artificial
  primer
tcctcggagaatggctcctg

SEQ ID NO: 29 - DNA, 20 bp, Artificial
  primer
ggcaggttgatgggaactgg

SEQ ID NO: 30 - DNA, 20 bp, Artificial
  primer
aaccagggtccccatcctgt

SEQ ID NO: 31 - DNA, 20 bp, Artificial
  primer
tgggctggtttcaatgctga

SEQ ID NO: 32 - DNA, 20 bp, Artificial
  primer
gtgtggccatggctggagta

SEQ ID NO: 33 - DNA, 20 bp, Artificial
  primer
tgttcctctgctgccactcg

SEQ ID NO: 34 - DNA, 20 bp, Artificial
  primer
acccagccactcccaccata

SEQ ID NO: 35 - DNA, 20 bp, Artificial
  primer
aagggcatggctatcccaca

SEQ ID NO: 36 - DNA, 38 bp, Artificial
  primer
tcgaggtaccgggagtaattttcaatccttgaggcaga

SEQ ID NO: 37 - DNA, 38 bp, Artificial
  primer
tcgactcgagtggcactgaccccttaattacgtacaga

SEQ ID NO: 38 - DNA, 37 bp, Artificial
  primer
tcgagtcgacaaagatttgcatccttggccatgactc

SEQ ID NO: 39 - DNA, 40 bp, Artificial
  primer
tcgagcggccgccatcagtgtacaccacaatcccatctgt

SEQ ID NO: 40 - DNA, 38 bp, Artificial
  primer
tcgaggtaccaagaacaagcttcagaacacagccagac

SEQ ID NO: 41 - DNA, 39 bp, Artificial
  primer
tcgactcgagaacttgtcacacagatcctactggaggtg

SEQ ID NO: 42 - DNA, 39 bp, Artificial
  primer
tcgagtcgacccacagactgaagcaattgacctcaaaag

SEQ ID NO: 43 - DNA, 40 bp, Artificial
  primer
tcgagcggccgcaaagcagttatccgctatttgggacctt

SEQ ID NO: 44 - DNA, 28 bp, Artificial
  primer
catgcacatttgcttacacacagaggtt

SEQ ID NO: 45 - DNA, 28 bp, Artificial
  primer
atctgggcactggggtacaactgttaat

SEQ ID NO: 46 - DNA, 29 bp, Artificial
  primer
ctgagaagagtcattgtttatggtagact

SEQ ID NO: 47 - DNA, 28 bp, Artificial
  primer
atccccatgtgtatcactggcaaactgt

SEQ ID NO: 48 - DNA, 28 bp, Artificial
  primer
ggggaataaacaccctttccaaatcctc

SEQ ID NO: 49 - DNA, 28 bp, Artificial
  primer
accaagtaaccgatcaaaccaacccttg

SEQ ID NO: 50 - DNA, 28 bp, Artificial
  primer
tgagaacacaggggtctccattctgact

SEQ ID NO: 51 - DNA, 28 bp, Artificial
  primer
acaatcaacagcatccccatctctgaag

SEQ ID NO: 52 - DNA, 28 bp, Artificial
  primer
gacgtgctacttccatttgtcacgtcct

SEQ ID NO: 53 - DNA, 28 bp, Artificial
  primer
tggtcactgaagctttccatctgctctt

SEQ ID NO: 54 - DNA, 20 bp, Artificial
  primer
agctcagagacacctctcca

SEQ ID NO: 55 - DNA, 25 bp, Artificial
  primer
ctgtattaggatacttggctattga

SEQ ID NO: 56 - DNA, 25 bp, Artificial
  primer
tatcaagggggtgtcggaaatcgtg

SEQ ID NO: 57 - DNA, 25 bp, Artificial
  primer
actgggcctgggagaacctgagact

SEQ ID NO: 58 - DNA, 22 bp, Artificial
  primer
aggtgctgctgggtggtcaagt

SEQ ID NO: 59 - DNA, 23 bp, Artificial
  primer
gctcctgcaaatgtctcctgtca

SEQ ID NO: 60 - DNA, 24 bp, Artificial
  primer
cttacccaggctccaggctctatt

SEQ ID NO: 61 - DNA, 25 bp, Artificial
  primer
ctctacctccctaccccatcatcac

SEQ ID NO: 62 - DNA, 20 bp, Artificial
  primer
tggaaggtggataacgccct

SEQ ID NO: 63 - DNA, 22 bp, Artificial
  primer
tcattctcctccaacattagca

SEQ ID NO: 64 - DNA, 20 bp, Artificial
  primer
agtcagggcattagcagtgc

SEQ ID NO: 65 - DNA, 20 bp, Artificial
  primer
gctgctgatggtgagagtga

SEQ ID NO: 66 - DNA, 20 bp, Artificial
  primer
ctctcctgcagggccagtca

SEQ ID NO: 67 - DNA, 22 bp, Artificial
  primer
tgctgatggtgagagtgaactc

SEQ ID NO: 68 - DNA, 25 bp, Artificial
  primer
ctctaactgaatcaagggaatgaac

SEQ ID NO: 69 - DNA, 24 bp, Artificial
  primer
agcagtttgagtttaggatgaagg

SEQ ID NO: 70 - DNA, 26 bp, Artificial
  primer
catcgccttctatcgccttcttgacg

SEQ ID NO: 71 - DNA, 28 bp, Artificial
  primer
atctgcacgagactagtgagacgtgcta

SEQ ID NO: 72 - DNA, 28 bp, Artificial
  primer
agcaattagggcctgtgcatctcacttt

SEQ ID NO: 73 - DNA, 28 bp, Artificial
  primer
ccagctcattcctcccactcatgatcta

SEQ ID NO: 74 - DNA, 28 bp, Artificial
  primer
catctggagtcctattgacatcgccagt

SEQ ID NO: 75 - DNA, 28 bp, Artificial
  primer
cttattcctccttctgcccacccttcat

SEQ ID NO: 76 - DNA, 24 bp, Artificial
  primer
agcactttacgcatcccagcatgt

SEQ ID NO: 77 - DNA, 24 bp, Artificial
  primer
ccaagagagtagtcgtgcccctca

SEQ ID NO: 78 - DNA, 20 bp, Artificial
  primer
cccactttaccgtgctcatt

SEQ ID NO: 79 - DNA, 20 bp, Artificial
  primer
atgaaggtccgtgactttgg

SEQ ID NO: 80 - DNA, 25 bp, Artificial
  primer
accccaaaggccaaactctccactc

SEQ ID NO: 81 - DNA, 24 bp, Artificial
  primer
cacttgtactccttgccattcagc

SEQ ID NO: 82 - DNA, 20 bp, Artificial
  primer
agtgagataagcagtggatg

SEQ ID NO: 83 - DNA, 20 bp, Artificial
  primer
cttgtgctactcccatcact

SEQ ID NO: 84 - DNA, 20 bp, Artificial
  primer
aggccagcatctgcgaggat

SEQ ID NO: 85 - DNA, 20 bp, Artificial
  primer
gtggcagcaagtagacatcg

SEQ ID NO: 86 - DNA, 28 bp, Artificial
  primer
cctattggcgttactatgggaacatacg

SEQ ID NO: 87 - DNA, 28 bp, Artificial
  primer
cctgccttcttgtttcagctctcaactg

SEQ ID NO: 88 - DNA, 28 bp, Artificial
  primer
gacgtgctacttccatttgtcacgtcct

SEQ ID NO: 89 - DNA, 28 bp, Artificial
  primer
atccccatgtgtatcactggcaaactgt

SEQ ID NO: 90 - DNA, 28 bp, Artificial
  primer
acactttagtccctgtcccctcaacgag

SEQ ID NO: 91 - DNA, 28 bp, Artificial
  primer
tgcaggtatctgttggtgtccctgtttt

SEQ ID NO: 92 - DNA, 28 bp, Artificial
  primer
gacgtgctacttccatttgtcacgtcct

SEQ ID NO: 93 - DNA, 28 bp, Artificial
  primer
agcagagctcgtttagtgaaccgtcaga

SEQ ID NO: 94 - DNA, 28 bp, Artificial
  primer
ctgtcctatccttgcagctgtcttccag

SEQ ID NO: 95 - DNA, 25 bp, Artificial
  primer
agatctcttgagcccagcagtttga

SEQ ID NO: 96 - DNA, 24 bp, Artificial
  primer
tgaagttagccggggatacagacg

SEQ ID NO: 97 - DNA, 20 bp, Artificial
  primer
aacggcagccaaaccaaaga

SEQ ID NO: 98 - DNA, 20 bp, Artificial
  primer
accaggactggctgggcata

SEQ ID NO: 99 - DNA, 20 bp, Artificial
  primer
agtctgcgctgacccaggaa

SEQ ID NO: 100 - DNA, 20 bp, Artificial
  primer
ttgagccagagaagcggtca

SEQ ID NO: 101 - DNA, 20 bp, Artificial
  primer
tccacttgggggtctgcatt

SEQ ID NO: 102 - DNA, 20 bp, Artificial
  primer
tggtgctgagcagctgtgtg

SEQ ID NO: 103 - DNA, 20 bp, Artificial
  primer
tgggacttaggtgggccaga

SEQ ID NO: 104 - DNA, 20 bp, Artificial
  primer
gcctccccaagagcctgaat

SEQ ID NO: 105 - DNA, 25 bp, Artificial
  primer
tgtcctgggctcctgtcctgctcat

SEQ ID NO: 106 - DNA, 20 bp, Artificial
  primer
ggcggcgactccaccctctt

SEQ ID NO: 107 - DNA, 22 bp, Artificial
  primer
cactgcctgcccgctgctggta

SEQ ID NO: 108 - DNA, 21 bp, Artificial
  primer
gggcggggaagtgggggagag

SEQ ID NO: 109 - DNA, 25 bp, Artificial
  primer
agccccaagaacccagccgatgtga

SEQ ID NO: 110 - DNA, 25 bp, Artificial
  primer
ggcagagggagtgtggggtgttgtg

SEQ ID NO: 111 - DNA, 20 bp, Artificial
  primer
atcatctgctcgctctctcc

SEQ ID NO: 112 - DNA, 20 bp, Artificial
  primer
cacatctgtagtggctgtgg

SEQ ID NO: 113 - DNA, 20 bp, Artificial
  primer
accagcgcgtcatcatcaag

SEQ ID NO: 114 - DNA, 20 bp, Artificial
  primer
atcgccagcctcaccatttc

SEQ ID NO: 115 - DNA, 22 bp, Artificial
  primer
ggagaccaccaaaccctccaaa

SEQ ID NO: 116 - DNA, 22 bp, Artificial
  primer
gagagttggagaaggggtgact

SEQ ID NO: 117 - DNA, 20 bp, Artificial
  primer
acctagagggtctcacctcc

SEQ ID NO: 118 - DNA, 19 bp, Artificial
  primer
ccctggacatcaagaatgg

SEQ ID NO: 119 - DNA, 20 bp, Artificial
  primer
cctcaggttgggcaggaaga

SEQ ID NO: 120 - DNA, 23 bp, Artificial
  primer
gacctaggaacagtcagcacggg

SEQ ID NO: 121 - DNA, 40 bp, Artificial
  primer
tcgagcggccgctctaagtcagggaaagatccccttcttg

SEQ ID NO: 122 - DNA, 38 bp, Artificial
  primer
tcgagtcgacgaccatgaagatggtccaactaaagcaa

SEQ ID NO: 123 - DNA, 40 bp, Artificial
  primer
tcgaatcgatcactgctctttctttagttacatgcagccc

SEQ ID NO: 124 - DNA, 38 bp, Artificial
  primer
tcgaatcgatattcttgccaagctactcttccgagcta

SEQ ID NO: 125 - DNA, 28 bp, Artificial
  primer
ctcttcagcaatatcacgggtagccaac

SEQ ID NO: 126 - DNA, 28 bp, Artificial
  primer
tgcttgcattgtatgtctggctattctg

SEQ ID NO: 127 - DNA, 20 bp, Artificial
  primer
tgctcaggtagtggttgtcg